European Patent Specification EP 4 041 908 B1, published September 20, 2023. Title: MICROORGANISM CAPTURE FROM ANTIMICROBIAL-CONTAINING SOLUTION. Applicant: Momentum Bioscience Ltd. The sequence listing filed with the application follows.

SEQUENCE LISTING (146 sequences)

SEQ ID NO: 1 - DNA, 20 bp, Artificial Sequence
  Probe or primer sequence
gaaggyccaaarggtggwcc

SEQ ID NO: 2 - DNA, 23 bp, Artificial Sequence
  Probe or primer sequence
gawccaccmgaraatctrccrtc

SEQ ID NO: 3 - DNA, 26 bp, Artificial Sequence
  Probe or primer sequence
gawggyttcaacatttcyggcatacc

SEQ ID NO: 4 - DNA, 18 bp, Artificial Sequence
  Probe or primer sequence
tcccttgttggccgattt

SEQ ID NO: 5 - DNA, 22 bp, Artificial Sequence
  Probe or primer sequence
taccgtcgataatgccttcttt

SEQ ID NO: 6 - DNA, 22 bp, Artificial Sequence
  Probe or primer sequence
aatcttgcagagggtgtcttag

SEQ ID NO: 7 - DNA, 19 bp, Artificial Sequence
  Probe or primer sequence
gggtcgcctgtgacaatag

SEQ ID NO: 8 - DNA, 21 bp, Artificial Sequence
  Probe or primer sequence
cagtaaatagggctggcttga

SEQ ID NO: 9 - DNA, 22 bp, Artificial Sequence
  Probe or primer sequence
ccttctgtaccgttggtgatac

SEQ ID NO: 10 - DNA, 20 bp, Artificial Sequence
  Probe or primer sequence
tgcctcgtcgtttgacatta

SEQ ID NO: 11 - DNA, 21 bp, Artificial Sequence
  Probe or primer sequence
gtacttaccggatggcttgaa

SEQ ID NO: 12 - DNA, 20 bp, Artificial Sequence
  Probe or primer sequence
cattgccactggtggttcta

SEQ ID NO: 13 - DNA, 22 bp, Artificial Sequence
  Probe or primer sequence
gatggcttgaagtcggctaata

SEQ ID NO: 14 - DNA, 20 bp, Artificial Sequence
  Probe or primer sequence
ccaggttctgctgttggtaa

SEQ ID NO: 15 - DNA, 22 bp, Artificial Sequence
  Probe or primer sequence
ccaaagcagtgatgaaggaatg

SEQ ID NO: 16 - DNA, 23 bp, Artificial Sequence
  Probe or primer sequence
gttctgctgttggtaaaatcact

SEQ ID NO: 17 - DNA, 22 bp, Artificial Sequence
  Probe or primer sequence
caaagcagtgatgaaggaatgt

SEQ ID NO: 18 - DNA, 21 bp, Artificial Sequence
  Probe or primer sequence
gccatgggaagacacaataga

SEQ ID NO: 19 - DNA, 23 bp, Artificial Sequence
  Probe or primer sequence
tcttgtcggcaatagctggatta

SEQ ID NO: 20 - DNA, 19 bp, Artificial Sequence
  Probe or primer sequence
gtggtggaagcaagagtaa

SEQ ID NO: 21 - DNA, 22 bp, Artificial Sequence
  Probe or primer sequence
gcttctcttccaaagtgatttg

SEQ ID NO: 22 - DNA, 23 bp, Artificial Sequence
  Probe or primer sequence
ttcaagccatctggtaagtatgt

SEQ ID NO: 23 - DNA, 22 bp, Artificial Sequence
  Probe or primer sequence
cagttaaggcgtcaccgtataa

SEQ ID NO: 24 - DNA, 20 bp, Artificial Sequence
  Probe or primer sequence
taaggccgaatggaaacctc

SEQ ID NO: 25 - DNA, 20 bp, Artificial Sequence
  Probe or primer sequence
acaaccttgggaggcattag

SEQ ID NO: 26 - DNA, 22 bp, Artificial Sequence
  Probe or primer sequence
gcctctcaggctatgttgtatg

SEQ ID NO: 27 - DNA, 20 bp, Artificial Sequence
  Probe or primer sequence
accagaccaccaacaagaac

SEQ ID NO: 28 - DNA, 22 bp, Artificial Sequence
  Probe or primer sequence
gacggtatctcgatgggtacta

SEQ ID NO: 29 - DNA, 21 bp, Artificial Sequence
  Probe or primer sequence
atcgtagtgttgtgccatcat

SEQ ID NO: 30 - DNA, 22 bp, Artificial Sequence
  Probe or primer sequence
atgggttacggcttaggtaaag

SEQ ID NO: 31 - DNA, 22 bp, Artificial Sequence
  Probe or primer sequence
tctggaacaatatggccgatta

SEQ ID NO: 32 - DNA, 22 bp, Artificial Sequence
  Probe or primer sequence
ggtggtatgtacactgccaata

SEQ ID NO: 33 - DNA, 20 bp, Artificial Sequence
  Probe or primer sequence
ccgaaactgctggagatgat

SEQ ID NO: 34 - DNA, 21 bp, Artificial Sequence
  Probe or primer sequence
tggtttcaaggacgaggattt

SEQ ID NO: 35 - DNA, 23 bp, Artificial Sequence
  Probe or primer sequence
cagaatctgcacatgccttattt

SEQ ID NO: 36 - DNA, 20 bp, Artificial Sequence
  Probe or primer sequence
gcggttctcacggtttctta

SEQ ID NO: 37 - DNA, 22 bp, Artificial Sequence
  Probe or primer sequence
ggcaagttcttcttcggataca

SEQ ID NO: 38 - DNA, 22 bp, Artificial Sequence
  Probe or primer sequence
ggaagaggccagagttgaaata

SEQ ID NO: 39 - DNA, 20 bp, Artificial Sequence
  Probe or primer sequence
cctttggaggcatcagagac

SEQ ID NO: 40 - DNA, 22 bp, Artificial Sequence
  Probe or primer sequence
gttcacgacggagatgagattg

SEQ ID NO: 41 - DNA, 22 bp, Artificial Sequence
  Probe or primer sequence
ggagaccacagcttctttcttt

SEQ ID NO: 42 - DNA, 20 bp, Artificial Sequence
  Probe or primer sequence
tcgatcgtgacccaggataa

SEQ ID NO: 43 - DNA, 22 bp, Artificial Sequence
  Probe or primer sequence
gaccaccatacacttccaactc

SEQ ID NO: 44 - DNA, 22 bp, Artificial Sequence
  Probe or primer sequence
gtgacccaggataagtctcaag

SEQ ID NO: 45 - DNA, 20 bp, Artificial Sequence
  Probe or primer sequence
ggtttcctgaccaccataca

SEQ ID NO: 46 - DNA, 22 bp, Artificial Sequence
  Probe or primer sequence
caaggctggattgaaaggaatg

SEQ ID NO: 47 - DNA, 21 bp, Artificial Sequence
  Probe or primer sequence
acatctgggccatcactaaag

SEQ ID NO: 48 - DNA, 23 bp, Artificial Sequence
  Probe or primer sequence
ctcctctgtaggcgttgaaatta

SEQ ID NO: 49 - DNA, 22 bp, Artificial Sequence
  Probe or primer sequence
caagtcagccatcacgtactta

SEQ ID NO: 50 - DNA, 22 bp, Artificial Sequence
  Probe or primer sequence
caccggtaaggaaggaacatac

SEQ ID NO: 51 - DNA, 22 bp, Artificial Sequence
  Probe or primer sequence
ccagcctgtaaagcagtgataa

SEQ ID NO: 52 - DNA, 22 bp, Artificial Sequence
  Probe or primer sequence
gccaagatgttgttggaagaag

SEQ ID NO: 53 - DNA, 22 bp, Artificial Sequence
  Probe or primer sequence
ggcatttgctcaagttctcttt

SEQ ID NO: 54 - DNA, 20 bp, Artificial Sequence
  Probe or primer sequence
aacatgcctggtgtgcttat

SEQ ID NO: 55 - DNA, 22 bp, Artificial Sequence
  Probe or primer sequence
ggcataatggtaccaccgtaaa

SEQ ID NO: 56 - DNA, 24 bp, Artificial Sequence
  Probe or primer sequence
actggtaagacactcaaagagaac

SEQ ID NO: 57 - DNA, 22 bp, Artificial Sequence
  Probe or primer sequence
ggtttcaatgggttggacaaag

SEQ ID NO: 58 - DNA, 24 bp, Artificial Sequence
  Probe or primer sequence
gaggaggactttatcactgcttta

SEQ ID NO: 59 - DNA, 22 bp, Artificial Sequence
  Probe or primer sequence
tctgataacacacacggtcttt

SEQ ID NO: 60 - DNA, 21 bp, Artificial Sequence
  Probe or primer sequence
attgaacaagcactcctcgat

SEQ ID NO: 61 - DNA, 22 bp, Artificial Sequence
  Probe or primer sequence
ccttaaacccagtagcgtacaa

SEQ ID NO: 62 - DNA, 22 bp, Artificial Sequence
  Probe or primer sequence
gcacttctaacagacggaagat

SEQ ID NO: 63 - DNA, 21 bp, Artificial Sequence
  Probe or primer sequence
tgggacaatgtgaccaatcaa

SEQ ID NO: 64 - DNA, 22 bp, Artificial Sequence
  Probe or primer sequence
ggtaaagccatcagacacttga

SEQ ID NO: 65 - DNA, 23 bp, Artificial Sequence
  Probe or primer sequence
acctccagtggcaatgatataag

SEQ ID NO: 66 - DNA, 23 bp, Artificial Sequence
  Probe or primer sequence
catggtttacggtggtaccatta

SEQ ID NO: 67 - DNA, 22 bp, Artificial Sequence
  Probe or primer sequence
ccgtatgattggaaagcagaga

SEQ ID NO: 68 - DNA, 22 bp, Artificial Sequence
  Probe or primer sequence
caacagaattgacttgctcgtg

SEQ ID NO: 69 - DNA, 23 bp, Artificial Sequence
  Probe or primer sequence
cgcaaagtacctctcttgtatct

SEQ ID NO: 70 - DNA, 15 bp, Artificial Sequence
  Probe or primer sequence
scagggtgcttcsca

SEQ ID NO: 71 - DNA, 16 bp, Artificial Sequence
  Probe or primer sequence
tsgcrtcgtaccactg

SEQ ID NO: 72 - DNA, 25 bp, Artificial Sequence
  Probe or primer sequence
cagtatgggtacaaagggwatgmga

SEQ ID NO: 73 - DNA, 20 bp, Artificial Sequence
  Probe or primer sequence
ggtacsaagggwatgcgata

SEQ ID NO: 74 - DNA, 20 bp, Artificial Sequence
  Probe or primer sequence
ctgatgttcgcrtcrtacca

SEQ ID NO: 75 - DNA, 23 bp, Artificial Sequence
  Probe or primer sequence
tcyatcgaraccgtyatgggtgg

SEQ ID NO: 76 - DNA, 22 bp, Artificial Sequence
  Probe or primer sequence
gcgaagaaacggctttgaataa

SEQ ID NO: 77 - DNA, 23 bp, Artificial Sequence
  Probe or primer sequence
ttgtaccagacagacgaaatacc

SEQ ID NO: 78 - DNA, 24 bp, Artificial Sequence
  Probe or primer sequence
acctgcgccttgttcatatcctcc

SEQ ID NO: 79 - DNA, 21 bp, Artificial Sequence
  Probe or primer sequence
gcctcacagaggaggatatga

SEQ ID NO: 80 - DNA, 20 bp, Artificial Sequence
  Probe or primer sequence
atccagcaggtgcatgttac

SEQ ID NO: 81 - DNA, 24 bp, Artificial Sequence
  Probe or primer sequence
ttcgtctgtctggtacaacggcaa

SEQ ID NO: 82 - DNA, 23 bp, Artificial Sequence
  Probe or primer sequence
aggcctcacagaggaggatatga

SEQ ID NO: 83 - DNA, 21 bp, Artificial Sequence
  Probe or primer sequence
gtaccaagggaatgcgatact

SEQ ID NO: 84 - DNA, 21 bp, Artificial Sequence
  Probe or primer sequence
gatactgatgttcgcgtcgta

SEQ ID NO: 85 - DNA, 23 bp, Artificial Sequence
  Probe or primer sequence
tccatcgaaaccgtcatgggtgg

SEQ ID NO: 86 - DNA, 20 bp, Artificial Sequence
  Probe or primer sequence
ctggtgtgccaccgatatta

SEQ ID NO: 87 - DNA, 21 bp, Artificial Sequence
  Probe or primer sequence
attgctgactctgtcggtatc

SEQ ID NO: 88 - DNA, 24 bp, Artificial Sequence
  Probe or primer sequence
agacaccgttcctggctgatttga

SEQ ID NO: 89 - DNA, 23 bp, Artificial Sequence
  Probe or primer sequence
gctataccaaacggaggagatac

SEQ ID NO: 90 - DNA, 19 bp, Artificial Sequence
  Probe or primer sequence
cttcccaggccatgcttta

SEQ ID NO: 91 - DNA, 24 bp, Artificial Sequence
  Probe or primer sequence
accgaggaggacatgaacaaagct

SEQ ID NO: 92 - DNA, 22 bp, Artificial Sequence
  Probe or primer sequence
ctataccaaacggaggagatac

SEQ ID NO: 93 - DNA, 22 bp, Artificial Sequence
  Probe or primer sequence
gttcaagacggcgatgttattc

SEQ ID NO: 94 - DNA, 20 bp, Artificial Sequence
  Probe or primer sequence
gcaacccagttctcctttct

SEQ ID NO: 95 - DNA, 24 bp, Artificial Sequence
  Probe or primer sequence
atgccgttgcgaacactttgtctg

SEQ ID NO: 96 - DNA, 22 bp, Artificial Sequence
  Probe or primer sequence
ggtatgcctgaaatgctcaaac

SEQ ID NO: 97 - DNA, 21 bp, Artificial Sequence
  Probe or primer sequence
ccatgagaacctccgctaaat

SEQ ID NO: 98 - DNA, 24 bp, Artificial Sequence
  Probe or primer sequence
agtttgatcatgggcgctggtcta

SEQ ID NO: 99 - DNA, 22 bp, Artificial Sequence
  Probe or primer sequence
acactttgtctgtggacgtatc

SEQ ID NO: 100 - DNA, 20 bp, Artificial Sequence
  Probe or primer sequence
gtaacagctcgggcgtattt

SEQ ID NO: 101 - DNA, 25 bp, Artificial Sequence
  Probe or primer sequence
tcaaggtcactcacggaacattgct

SEQ ID NO: 102 - DNA, 20 bp, Artificial Sequence
  Probe or primer sequence
cgtcgaaagcggttctatca

SEQ ID NO: 103 - DNA, 22 bp, Artificial Sequence
  Probe or primer sequence
ggtttgagcatttcaggcatac

SEQ ID NO: 104 - DNA, 24 bp, Artificial Sequence
  Probe or primer sequence
tgttgtcttgaggtaccttggccc

SEQ ID NO: 105 - DNA, 23 bp, Artificial Sequence
  Probe or primer sequence
tcgacccagtatgatggtttatg

SEQ ID NO: 106 - DNA, 21 bp, Artificial Sequence
  Probe or primer sequence
tttggccttcttggaggtatc

SEQ ID NO: 107 - DNA, 24 bp, Artificial Sequence
  Probe or primer sequence
cggagaggtgctcgacattgtgtc

SEQ ID NO: 108 - DNA, 16 bp, Artificial Sequence
  Probe or primer sequence
tacgggaggcagcagt

SEQ ID NO: 109 - DNA, 16 bp, Artificial Sequence
  Probe or primer sequence
tattaccgcggctgct

SEQ ID NO: 110 - DNA, 28 bp, Artificial Sequence
  Probe or primer sequence
ccgcagaataagcaccggctaactccgt

SEQ ID NO: 111 - DNA, 30 bp, Artificial Sequence
  Probe or primer sequence
cctaaccagaaagccacggctaactacgtg

SEQ ID NO: 112 - DNA, 19 bp, Artificial Sequence
  Probe or primer sequence
caacgcgaagaaccttacc

SEQ ID NO: 113 - DNA, 18 bp, Artificial Sequence
  Probe or primer sequence
acgtcatccccaccttcc

SEQ ID NO: 114 - DNA, 21 bp, Artificial Sequence
  Probe or primer sequence
acgacaaccatgcaccacctg

SEQ ID NO: 115 - DNA, 20 bp, Artificial Sequence
  Probe or primer sequence
acgacagccatgcagcacct

SEQ ID NO: 116 - DNA, 24 bp, Artificial Sequence
  Probe or primer sequence
cggcggtacacctgctgttatgaa

SEQ ID NO: 117 - DNA, 28 bp, Artificial Sequence
  Probe or primer seqeuence
tgcttgattgtggatgtagcaaatgtcc

SEQ ID NO: 118 - DNA, 24 bp, Artificial Sequence
  Probe or primer sequence
aattgcatggctttcaagccagcc

SEQ ID NO: 119 - DNA, 24 bp, Artificial Sequence
  Probe or primer sequence
attagccgacttcaagccatccgg

SEQ ID NO: 120 - DNA, 26 bp, Artificial Sequence
  Probe or primer sequence
tgcctcgtcgtttgacattaccatca

SEQ ID NO: 121 - DNA, 30 bp, Artificial Sequence
  Probe or primer sequence
aggtacttacttcaagggtaaagctagagt

SEQ ID NO: 122 - DNA, 25 bp, Artificial Sequence
  Probe or primer sequence
tactatcttgccagggtctcccaca

SEQ ID NO: 123 - DNA, 24 bp, Artificial Sequence
  Probe or primer sequence
tcctgctattgctgacaagattga

SEQ ID NO: 124 - DNA, 24 bp, Artificial Sequence
  Probe or primer sequence
aggtcggtggtactcaaagtgtca

SEQ ID NO: 125 - DNA, 26 bp, Artificial Sequence
  Probe or primer sequence
tgctaagttagtctctaatgcctccc

SEQ ID NO: 126 - DNA, 24 bp, Artificial Sequence
  Probe or primer sequence
tcagcaaagcgcaagttggtgttg

SEQ ID NO: 127 - DNA, 30 bp, Artificial Sequence
  Probe or primer sequence
agagaaattatcgcagactctttcgagact

SEQ ID NO: 128 - DNA, 24 bp, Artificial Sequence
  Probe or primer sequence
attctctggcggttctcacggttt

SEQ ID NO: 129 - DNA, 24 bp, Artificial Sequence
  Probe or primer sequence
acccaagacttctgaggctgaagc

SEQ ID NO: 130 - DNA, 24 bp, Artificial Sequence
  Probe or primer sequence
tggttcttgctggtggtctggaaa

SEQ ID NO: 131 - DNA, 24 bp, Artificial Sequence
  Probe or primer sequence
agaagctttcgaaggcggtccaat

SEQ ID NO: 132 - DNA, 26 bp, Artificial Sequence
  Probe or primer sequence
cctctcttatatttcaactctggcct

SEQ ID NO: 133 - DNA, 26 bp, Artificial Sequence
  Probe or primer sequence
tgcttgtctcggaagaaattctcgct

SEQ ID NO: 134 - DNA, 24 bp, Artificial Sequence
  Probe or primer sequence
tgcttcgcaagccatgttgtatgc

SEQ ID NO: 135 - DNA, 27 bp, Artificial Sequence
  Probe or primer sequence
accgttggtgataccatcagaaactcc

SEQ ID NO: 136 - DNA, 24 bp, Artificial Sequence
  Probe or primer sequence
tctgacagcactccattgttggct

SEQ ID NO: 137 - DNA, 24 bp, Artificial Sequence
  Probe or primer sequence
aaaggctagagtgtttgacgccga

SEQ ID NO: 138 - DNA, 25 bp, Artificial Sequence
  Probe or primer sequence
tgcttgatggtgaccagatgactgt

SEQ ID NO: 139 - DNA, 25 bp, Artificial Sequence
  Probe or primer sequence
aaggtctgttgtgtctacccatggc

SEQ ID NO: 140 - DNA, 22 bp, Artificial Sequence
  Probe or primer sequence
atatcctggccctcaggcaagc

SEQ ID NO: 141 - DNA, 24 bp, Artificial Sequence
  Probe or primer sequence
tcgcccttcttgatttctccagcc

SEQ ID NO: 142 - DNA, 22 bp, Artificial Sequence
  Probe or primer sequence
tgtcaccgaggatgtgtcgcag

SEQ ID NO: 143 - DNA, 23 bp, Artificial Sequence
  Probe or primer sequence
tttctggtggatcccacggtttc

SEQ ID NO: 144 - DNA, 27 bp, Artificial Sequence
  Probe or primer sequence
cccgtgacatcatgaccaagaaatcgt

SEQ ID NO: 145 - DNA, 24 bp, Artificial Sequence
  Probe or primer sequence
tggccatgggtagacacaacagac

SEQ ID NO: 146 - DNA, 24 bp, Artificial Sequence
  Probe or primer sequence
aagaaagaagtggctgcctcctga